European Patent Application EP 4 389 878 A1, published June 26, 2024. Title: Method of producing gene-modified T cells population. Applicant: KEIO UNIVERSITY. Application JP. The sequence listing filed with the application follows.

SEQUENCE LISTING (1 sequence)

SEQ ID NO: 1 - DNA, 1464 bp, synthetic construct
  misc_feature 1..1464: note = Chimeric Antigen Receptror Gene
  source 1..1464: mol_type = other DNA
atggccttaccagtgaccgccttgctcctgccgctggccttgctgctccacgccgccaggccggcggtgacgttggacgagtccgggggcggcctccagacgcccggaagagcgctcagcctcgtctgtaaggcctccgggttcaccttcagccgttacgccatgtactgggtgcgacaggcgcccggcaaggggctggagttcgtcgctggtattggcaacactggtagatacacaggctacgggtcggcggtgaagggccgtgccaccatctcgagggacagcgggcagagcacagtgaggctgcaactgaacaacctcagggctgaggacaccggcaactactactgcgccaaaagtgttagtccttactgttgtgatgctgctgacatcgacgcatggggccacgggaccgaagtcatcgtctcctccggcggtggcggatcaggtggcggtggaagtggcggtggtgggtctgctagcactcagccgtcctcggtgtcagcaaacccaggagaaaccgtcaagatcacctgctccgggggtagcagtggctatgcttatggctggtaccagcagaagtctcctggcagtgcccctgtcactctgctctatagcaacaacaacagaccctcggacatcccttcacgattctccggttccaaatccggctccacagccacattaaccatcactggggtccaagccgaggacgaggctgtctatttctgtgggagtgtagacagcagcagttatgctggtatatttggggccgggacaaccctgaccgtcctagcggccgcaattgaagttatgtatcctcctccttacctagacaatgagaagagcaatggaaccattatccatgtgaaagggaaacacctttgtccaagtcccctatttcccggaccttctaagcccttttgggtgctggtggtggttggtggagtcctggcttgctatagcttgctagtaacagtggcctttattattttctgggtgaggagtaagaggagcaggctcctgcacagtgactacatgaacatgactccccgccgccccgggcccacccgcaagcattaccagccctatgccccaccacgcgacttcgcagcctatcgctccagagtgaagttcagcaggagcgcagacgcccccgcgtaccagcagggccagaaccagctctataacgagctcaatctaggacgaagagaggagtacgatgttttggacaagagacgtggccgggaccctgagatggggggaaagccgagaaggaagaaccctcaggaaggcctgtacaatgaactgcagaaagataagatggcggaggcctacagtgagattgggatgaaaggcgagcgccggaggggcaaggggcacgatggcctttaccagggtctcagtacagccaccaaggacacctacgacgcccttcacatgcaggccctgccccctcgctaa